European Patent Application EP 4 388 875 A1, published June 26, 2024. Title: EFFECT OF FLAVONOID GLYCOSIDE IN RESISTANCE OF RICE TO WEEDS. Applicant: INSTITUTE OF BOTANY, THE CHINESE ACADEMY OF SCIENCE. The sequence listing filed with the application follows.

SEQUENCE LISTING (2 sequences)

SEQ ID NO: 1 - protein, 431 aa, Artificial sequence
  Synthesized
MDASPLHVVVFPWLAFGHLLPALELAGRLASRGLRVSFVSTPRNIARLRRPCPSVEFVELPLPRVDGLPDGAEATTDVPDHMSSALWKASDGLTAPFSAFLDAAAAAGNKVDWLILDGMLSWAAASAADRKVPCVLMMPYTATACAHFGVPDEARDADRFPSAIARRFVSAFRSSELLAVRSCVEFEPESVPLLSNIFGKPVVPIGLLPPPQVDGDGDGDTALMSSWLDRQPPKSVVYVALGSEAPLTAEQRRELALGLELSGAPFLWALRKPHGGDDDGGLLPPGFEERTRGRGMVKTEWVPQLKILAHAAVGAFLTHCGHSSVIEGLRFGHPLVMLPLFLDQFTNASYLEGARGVGVQVARDGEHGGAFDRDGVAAAVRAAVVDEESKKALAANAGKMGEVVADTECHERCIDAFIQQLRSYTTTRTGY

SEQ ID NO: 2 - DNA, 1296 bp, Artificial sequence
  Synthesized
atggatgcctccccgctgcacgtcgtcgtcttcccgtggctcgcgttcggccacctcctccctgccctcgagctcgccggccgcctggcctcgcgcggcctccgcgtgtccttcgtctccaccccgcgcaacatcgctcgcctccgccgcccgtgcccgtccgtcgagttcgtcgagctgccgctcccgcgcgtcgacggcctccccgacggcgccgaggccaccaccgacgtccccgatcacatgtcatccgctctctggaaggcctccgatgggctcaccgcgcccttctccgccttcctcgacgccgccgccgccgcggggaacaaggtcgactggctcatcctcgacggcatgctttcctgggccgccgcctccgccgccgaccgcaaggttccctgcgtcctcatgatgccgtacacggcgacggcgtgcgcgcatttcggcgtgccggatgaggcgcgggacgccgaccgtttcccctccgccatagcccggcggttcgtctcggccttccggagcagcgagcttctcgccgtgcggagctgcgtggagttcgagcccgagtcggtgcctctcctgtcgaacatcttcggcaagccggtcgtccccatcggccttctcccgccgccgcaggttgacggcgacggcgacggcgacacagctctcatgtcctcgtggctcgacaggcagccgcccaagtccgtcgtctacgtcgcgctcgggagcgaggcgccgctgaccgcggagcagcggcgcgagctggcgctcgggctggagctctccggcgcgcccttcctctgggccctgaggaagcctcacggcggcgacgacgacggcggcctcctgcctccgggattcgaggagcggacgcgcgggcgcgggatggtgaagacggagtgggtgccccagctcaagatcctggcgcacgccgccgtgggcgccttcctgacgcactgcggccacagctccgtcatcgaggggctccggttcggccatcctctcgtcatgctgccactgttcctcgaccagttcactaacgcgagctacttggaaggggcgagaggggttggggtgcaggtggccagggatggcgagcacggcggcgccttcgaccgggacggcgtcgccgcagccgtccgggccgccgtggtggatgaagagagcaagaaggcgctcgccgccaacgccgggaagatgggggaggtggtggccgacacggagtgtcacgagaggtgcatcgacgctttcattcagcagctcaggtcctatacaacgacaaggactggttattag